European Patent Application EP 4 541 895 A1, published April 23, 2025. Title: Detection Method of Test Substance Using Polynucleotide. Applicant: 国立大学法人東京農工大学. The sequence listing filed with the application follows.

SEQUENCE LISTING (10 sequences)

SEQ ID NO: 1 - DNA, 26 bp, synthetic construct
  misc_feature 1..26: note = SARS-CoV-2 RBD-binding aptamer
  source 1..26: mol_type = other DNA
ggggctgctcgggattgcggatatgg

SEQ ID NO: 2 - DNA, 51 bp, synthetic construct
  misc_feature 1..51: note = SARS-CoV-2 RBD-binding aptamer
  source 1..51: mol_type = other DNA
cagcaccgaccttgtgctttgggagtgctggtccaagggcgttaatggaca

SEQ ID NO: 3 - DNA, 67 bp, synthetic construct
  misc_feature 1..67: note = SARS-CoV-2 RBD-binding aptamer
  source 1..67: mol_type = other DNA
atccagagtgacgcagcatttcatcgggtccaaaaggggctgctcgggattgcggatatggacacgt

SEQ ID NO: 4 - DNA, 38 bp, synthetic construct
  misc_feature 1..38: note = SARS-CoV-2 RBD-binding aptamer
  source 1..38: mol_type = other DNA
cgggtccaaaaggggctgctcgggattgcggatatgga

SEQ ID NO: 5 - DNA, 36 bp, synthetic construct
  misc_feature 1..36: note = SARS-CoV-2 RBD-binding aptamer
  source 1..36: mol_type = other DNA
gggtccaaaaggggctgctcgggattgcggatatgg

SEQ ID NO: 6 - DNA, 32 bp, synthetic construct
  misc_feature 1..32: note = SARS-CoV-2 RBD-binding aptamer
  source 1..32: mol_type = other DNA
cgggtccaaaaggggctgctcgggattgcgga

SEQ ID NO: 7 - DNA, 30 bp, synthetic construct
  misc_feature 1..30: note = SARS-CoV-2 RBD-binding aptamer
  source 1..30: mol_type = other DNA
gggtccaaaaggggctgctcgggattgcgg

SEQ ID NO: 8 - DNA, 28 bp, synthetic construct
  misc_feature 1..28: note = SARS-CoV-2 RBD-binding aptamer
  source 1..28: mol_type = other DNA
aggggctgctcgggattgcggatatgga

SEQ ID NO: 9 - DNA, 31 bp, synthetic construct
  misc_feature 1..31: note = SARS-CoV-2 RBD-binding aptamer
  source 1..31: mol_type = other DNA
gcagcatttcatcgggtccaaaaggggctgc

SEQ ID NO: 10 - DNA, 29 bp, synthetic construct
  misc_feature 1..29: note = SARS-CoV-2 RBD-binding aptamer
  source 1..29: mol_type = other DNA
tcgggattgcggatatggacacgttatcc